European Patent Specification EP 3 775 281 B1, published March 5, 2025. Title: METHODS FOR PREDICTING THE RISK OF DEVELOPING PULMONARY COLONIZATION/INFECTION BY PSEUDOMONAS AERUGINOSA. Applicant: INSERM. The sequence listing filed with the application follows.

SEQUENCE LISTING (2 sequences)

SEQ ID NO: 1 - DNA, 20 bp, Artificial
  Primer sense
gtgtcttcgcccagcttact

SEQ ID NO: 2 - DNA, 18 bp, Artificial
  Primer antisense
aggatgcggcgggtttca